European Patent Application EP 4 509 133 A1, published February 19, 2025. Title: 암의 예방 또는 치료를 위한 ADP-리보오스 결합 펩티드 및 ADP-리보오스의 병용 요법. Applicant: 주식회사 펄스인마이어스. Application KR. The sequence listing filed with the application follows.

SEQUENCE LISTING (29 sequences)

SEQ ID NO: 1 - protein, 24 aa, synthetic construct
RRYTVQFTTMVQVNEETGNRRPVM

SEQ ID NO: 2 - protein, 26 aa, synthetic construct
FLYVADLENMVQYRRNEHGRRRKIKR

SEQ ID NO: 3 - protein, 25 aa, synthetic construct
RVYTIDFNSMQQINEDTGTARAIQR

SEQ ID NO: 4 - protein, 25 aa, synthetic construct
VPYIIDLQSMHQFRQDTGTMRPVRR

SEQ ID NO: 5 - protein, 25 aa, synthetic construct
FSYKIDFAEMKQMNLTTGKQRLIKR

SEQ ID NO: 6 - protein, 26 aa, synthetic construct
GRYDVHLGERMRYAVYWDELASEVRR

SEQ ID NO: 7 - protein, 25 aa, synthetic construct
APYIIDLQSMNQFRQDTGTLRPVRR

SEQ ID NO: 8 - protein, 25 aa, synthetic construct
APYIIDLPSWTQFRQDTGTMRAVRR

SEQ ID NO: 9 - protein, 25 aa, synthetic construct
FCYLIYFNSMSQMNRQTRRRRRLRR

SEQ ID NO: 10 - protein, 25 aa, synthetic construct
FSYVIDFNTMGQINRQTQRQRRVRR

SEQ ID NO: 11 - protein, 25 aa, synthetic construct
YNYTVNYTTHTQTNKTSSFCRSVRR

SEQ ID NO: 12 - protein, 24 aa, synthetic construct
WIWYWKNESGTWIQYGEEKDKRKN

SEQ ID NO: 13 - protein, 24 aa, synthetic construct
RHYTVNLNTYTATDTKGHSLSVQR

SEQ ID NO: 14 - protein, 19 aa, synthetic construct
TAYEASVCDYLEQQVARGN

SEQ ID NO: 15 - protein, 36 aa, synthetic construct
GRKKRRQRRRPQRRYTVQFTTMVQVNEETGNRRPVM

SEQ ID NO: 16 - protein, 43 aa, synthetic construct
RAGLQFPVGRLLRRLLRFLYVADLENMVQYRRNEHGRRRKIKR

SEQ ID NO: 17 - protein, 37 aa, synthetic construct
GRKKRRQRRRPQRVYTIDFNSMQQINEDTGTARAIQR

SEQ ID NO: 18 - protein, 37 aa, synthetic construct
GRKKRRQRRRPQVPYIIDLQSMHQFRQDTGTMRPVRR

SEQ ID NO: 19 - protein, 37 aa, synthetic construct
GRKKRRQRRRPQFSYKIDFAEMKQMNLTTGKQRLIKR

SEQ ID NO: 20 - protein, 38 aa, synthetic construct
GRKKRRQRRRPQGRYDVHLGERMRYAVYWDELASEVRR

SEQ ID NO: 21 - protein, 37 aa, synthetic construct
GRKKRRQRRRPQAPYIIDLQSMNQFRQDTGTLRPVRR

SEQ ID NO: 22 - protein, 37 aa, synthetic construct
GRKKRRQRRRPQAPYIIDLPSWTQFRQDTGTMRAVRR

SEQ ID NO: 23 - protein, 37 aa, synthetic construct
GRKKRRQRRRPQFCYLIYFNSMSQMNRQTRRRRRLRR

SEQ ID NO: 24 - protein, 37 aa, synthetic construct
GRKKRRQRRRPQFSYVIDFNTMGQINRQTQRQRRVRR

SEQ ID NO: 25 - protein, 37 aa, synthetic construct
GRKKRRQRRRPQYNYTVNYTTHTQTNKTSSFCRSVRR

SEQ ID NO: 26 - protein, 36 aa, synthetic construct
GRKKRRQRRRPQWIWYWKNESGTWIQYGEEKDKRKN

SEQ ID NO: 27 - protein, 36 aa, synthetic construct
GRKKRRQRRRPQRHYTVNLNTYTATDTKGHSLSVQR

SEQ ID NO: 28 - protein, 31 aa, synthetic construct
GRKKRRQRRRPQTAYEASVCDYLEQQVARGN

SEQ ID NO: 29 - protein, 38 aa, synthetic construct
GRKKRRQRRRPQFLYVADLENMVQYRRNEHGRRRKIKR